European Patent Application EP 4 116 709 A1, published January 11, 2023. Title: DETECTION METHOD FOR INSULIN AND DETECTION KIT FOR INSULIN. Applicant: Hiroshima University Terumo Kabushiki Kaisha. The sequence listing filed with the application follows.

SEQUENCE LISTING (4 sequences)

SEQ ID NO: 1 - protein, 436 aa, Artificial Sequence
  Artificially Synthesized Sequence
  BINDING (1)..(14)
METDTLLLWVLLLWVPGSTGDQLMHGKTQATSGTIQSMHGKTQATSGTIQSMHGKTQATSGTIQSMTFEDYLHNVVFVPRPSASSAGGSAGGSAGGSAGGSAGGSAGGSAGSGGLEHLYPGEVCPGMDIRNNLTRLHELENCSVIEGHLQILLMFKTRPEDFRDLSFPKLIMITDYLLLFRVYGLESLKDLFPNLTVIRGSRLFFNYALVIFEMVHLKELGLYNLMNITRGSVRIEKNNELCYLATIDWSRILDSVEDNYIVLNKDDNEECGDVCPGTAKGKTNCPATVINGQFVERCWTHSHCQKVCPTICKSHGCTAEGLCCHKECLGNCSEPDDPTKCVACRNFYLDGQCVETCPPPYYHFQDWRCVNFSFCQDLHFKCRNSRKPGCHQYVIHNNKCIPECPSGYTMNSSNLMCTPCLGPCPKSRTGHHHHHH

SEQ ID NO: 2 - DNA, 1290 bp, Artificial Sequence
  Artificially Synthesized Sequence
  protein_bind (199)..(246)
atggagacagacacactcctgctatgggtactgctgctctgggttccaggttccactggtgaccagcttatgcatgggaaaacacaagccacaagtggcaccattcagtctatgcatggtaagacccaggcaacgtcaggcacaatccagtcaatgcacggtaaaactcaggccacttccggcacaatacagagtatgacgtttgaggattacctccacaatgtcgtgtttgtgcccagaccaagtgctagctccgctggtggatcagctggaggttccgctggaggaagcgccggtggttctgccggagggagtgcaggcgggagcgcagggagcggagggctggaacatctgtacccaggagaagtctgccctggcatggacatccggaataacctgaccaggcttcacgagctggagaattgtagcgtgatcgaagggcacttgcagatcttgttgatgtttaaaactcgccctgaggatttccgggatctgtcttttcctaagctgatcatgattactgactacctgttgctgttccgcgtgtatgggctcgagtccctgaaggacctctttcccaatctgaccgtgattagagggagtcggctcttcttcaactacgcgctggtgattttcgagatggtccacctgaaggagcttgggctgtataacctgatgaacataacccgagggtctgtcaggatcgagaagaacaacgagctgtgctatctggccacaattgactggtcccgtatcctcgatagcgttgaggacaattacattgtccttaacaaggacgacaacgaagaatgtggcgatgtatgtcccggcactgccaaaggcaaaaccaactgccctgccacagttattaatggccagtttgtggaaagatgttggacccactcacactgtcagaaggtttgccccactatctgcaaatctcatggatgcactgcagaaggcctctgttgccataaggagtgtctgggcaattgttcagagcctgatgatcccacaaagtgcgtagcgtgccgaaatttctacctggacggacagtgtgttgaaacctgtccgccaccctactatcatttccaggattggcgctgtgtgaatttcagcttttgccaagacctccacttcaagtgcaggaactccaggaaaccaggctgccatcaatatgtgatccacaacaacaaatgcataccggaatgcccaagcggctatacgatgaattccagcaatctgatgtgcaccccatgtcttggaccttgtcccaagtctagaaccggt

SEQ ID NO: 3 - protein, 436 aa, Artificial Sequence
  Artificially Synthesized Sequence
  BINDING (387)..(428)
METDTLLLWVLLLWVPGSTGDQLMTFEDYLHNVVFVPRPSASSAGGSAGGSAGGSAGGSAGGSAGGSAGSGGLEHLYPGEVCPGMDIRNNLTRLHELENCSVIEGHLQILLMFKTRPEDFRDLSFPKLIMITDYLLLFRVYGLESLKDLFPNLTVIRGSRLFFNYALVIFEMVHLKELGLYNLMNITRGSVRIEKNNELCYLATIDWSRILDSVEDNYIVLNKDDNEECGDVCPGTAKGKTNCPATVINGQFVERCWTHSHCQKVCPTICKSHGCTAEGLCCHKECLGNCSEPDDPTKCVACRNFYLDGQCVETCPPPYYHFQDWRCVNFSFCQDLHFKCRNSRKPGCHQYVIHNNKCIPECPSGYTMNSSNLMCTPCLGPCPKSRMHGKTQATSGTIQSMHGKTQATSGTIQSMHGKTQATSGTIQSTGHHHHHH

SEQ ID NO: 4 - DNA, 1290 bp, Artificial Sequence
  Artificially Synthesized Sequence
  protein_bind (70)..(123)
atggagacagacacactcctgctatgggtactgctgctctgggttccaggttccactggtgaccagcttatgacctttgaggactatctgcacaatgtcgttttcgtgccacgaccctcagcctccagtgccggtggatccgctggagggtccgcaggcggaagcgccggcgggtcagctggtggaagtgctggtgggtctgctggcagcggcgggctggagcatctttatccaggcgaagtgtgtcccggaatggacatccgtaacaatctgaccagactgcacgaactcgagaactgctctgtcatcgaagggcatctccagattctgctgatgttcaaaacgaggcccgaagatttccgggacctgtcattccccaaactgatcatgattactgattatctgctcctctttcgcgtttacgggctggaatcccttaaagacctctttccaaatctgacagtgattcggggatctcgcttgttcttcaactatgcccttgtcatcttcgagatggtgcacttgaaggaactgggactctacaacttgatgaacataactagaggttccgtaagaatagagaagaataatgagctgtgctacttggcaaccatcgattggtcaaggatactggatagcgtcgaggacaactacatcgtgctgaacaaagacgataacgaggagtgtggggacgtttgcccaggcactgcaaagggcaagaccaattgccctgccacagtgattaatggccagtttgtggagagatgctggactcactcccattgccagaaagtctgtccaacgatctgtaaaagtcatggctgcacagccgagggactgtgctgccataaggaatgcctcgggaattgcagtgaacctgacgatcccaccaagtgtgttgcctgtcgcaacttttacctggatgggcaatgtgtagaaacttgtccgccaccctattaccatttccaggattggaggtgtgtgaacttcagcttttgccaagaccttcactttaaatgtaggaactcccggaagcctggctgccaccagtacgtgattcacaataacaagtgcattcctgagtgtccgtcagggtataccatgaatagcagcaatctgatgtgtacaccctgtctgggcccttgccctaagagccgaatgcacggaaagactcaggcaacaagtggcacaatccagagcatgcatggtaagacccaagcgacctctggtaccatccagtctatgcacggcaaaacacaggcgactagcggaacgattcagtctaccggt